European Patent Specification EP 3 641 748 B1, published November 29, 2023. Title: TREATING DISEASE AND PROMOTING WEIGHT LOSS BY INHIBITING THE TMA/FMO3/TMAO PATHWAY. Applicant: THE CLEVELAND CLINIC FOUNDATION. The sequence listing filed with the application follows.

SEQUENCE LISTING (7 sequences)

SEQ ID NO: 1 - DNA, 188 bp, Artificial sequence
  Synthetic
gaccatatagaagagggcagggccagcatttaccaatcggtcttcaccaactcttccaaagagatgatgtgtttccagacttcccctatcccgatgactttcccaacttcatgcatcacagcaagctccaagaatacatcacttcatttgccaaggaaaagaacctcctgaaatacatacagtttgag

SEQ ID NO: 2 - DNA, 20 bp, Artificial sequence
  Synthetic
tgggaaagtcatcgggatag

SEQ ID NO: 3 - DNA, 1125 bp, Escherichia coli str. K-12 substr. DH10B
atgagcaatctgagccctgactttgtactacccgaaaatttttgcgctaacccgcaagaggcgtggaccattcctgcccgtttttataccgatcagaacgcgtttgaacacgaaaaagagaacgtcttcgccaaaagctggatttgcgtcgctcacagcagcgaactggcgaatgccaatgattatgtgacgcgtgagatcattggcgaaagcatcgtgctggtacgcggtcgtgataaggttttgcgcgcgttctataacgtgtgtccgcaccgtggtcatcagttgttgagcggtgaaggaaaagcaaaaaatgtgattacctgcccgtatcacgcatgggcattcaaactcgatggcaacctggcccatgcacgtaactgcgaaaacgtcgccaatttcgatagcgacaaagcgcaactggttccggtgcgtctggaagaatatgccggattcgtcttcatcaacatggaccccaacgccaccagcgtagaagatcaattacccggcctgggcgcgaaagtgctggaagcctgcccggaagtccacgatctgaaactggcggcccgctttaccacccgcacgcctgccaactggaagaacattgtcgataactatctcgagtgctatcactgtggtccggcgcatccaggtttctccgactccgtacaggttgatcgttactggcacaccatgcacggtaactggacgctgcaatacggtttcgccaaaccgtccgaacagtcgtttaaatttgaagagggtacggatgcggcattccacggtttctggctgtggccgtgcacgatgctgaacgtcaccccgatcaaagggatgatgacggtcatttatgaattcccggtggattctgaaactaccctgcaaaactacgatatttacttcaccaatgaagagttaaccgacgagcaaaaatcgctgattgagtggtatcgcgatgtgttccgtccggaagatttacgtctggttgaaagcgtacagaaagggctgaaatcgcgtggctatcgtggtcaggggcgcatcatggccgacagtagcggtagtggcatttccgaacatggtatcgcccatttccataatctgctggcgcaggtgtttaaggactaa

SEQ ID NO: 4 - protein, 374 aa, Escherichia coli str. K-12 substr. DH10B
MSNLSPDFVLPENFCANPQEAWTIPARFYTDQNAFEHEKENVFAKSWICVAHSSELANANDYVTREIIGESIVLVRGRDKVLRAFYNVCPHRGHQLLSGEGKAKNVITCPYHAWAFKLDGNLAHARNCENVANFDSDKAQLVPVRLEEYAGFVFINMDPNATSVEDQLPGLGAKVLEACPEVHDLKLAARFTTRTPANWKNIVDNYLECYHCGPAHPGFSDSVQVDRYWHTMHGNWTLQYGFAKPSEQSFKFEEGTDAAFHGFWLWPCTMLNVTPIKGMMTVIYEFPVDSETTLQNYDIYFTNEELTDEQKSLIEWYRDVFRPEDLRLVESVQKGLKSRGYRGQGRIMADSSGSGISEHGIAHFHNLLAQVFKD

SEQ ID NO: 5 - DNA, 966 bp, Escherichia coli str. K-12 substr. DH10B
atgtcagactatcaaatgtttgaagtacaggtgagccaggttgaaccccttaccgaacaggtgaaacgcttcacgctggtggcaaccgatggcaaaccattacctgcgtttaccggaggaagtcacgtcattgtgcagatgagcgatggtgataaccagtacagcaatgcgtattcactactgagttcgccgcatgacacctcttgttatcagattgccgttcggctggaggaaaactcgcgcggcggttcccgctttttgcatcagcaggtaaaagtgggcgatcggttaacgatttcaacgcctaataacctgtttgcgctaattccctcagccagaaagcatctgtttatcgcgggcggtattggtatcacccctttcctgtcgcacatggcagagctgcaacacagcgacgtcgactggcagctacattactgctcgcgaaatccagaaagttgcgcatttcgtgatgagctagtccagcatccgcaggctgagaaagtccatttgcatcattcatcaaccggaacacgactggaattagcgcgattattggcggatatcgaacctggcacacacgtttatacctgtggccccgaggcgctaattgaagcggtaagaagtgaagctgcgcgtctggacatcgccgccgatacgctgcactttgagcaatttgctatcgaagacaaaaccggcgatgcatttaccctggtgcttgcccgttccggaaaagagtttgtggtgccggaagagatgactattttgcaggttattgaaaataataaagccgcgaaagtggaatgtttatgtcgtgaaggggtatgcggaacctgcgaaacagcaatactggaaggtgaagctgaccatcgggatcaatattttagcgatgaagagcgtgccagccagcaaagtatgttgatctgttgttcgcgtgcgaagggtaaacgcctggtgttggatttgtag

SEQ ID NO: 6 - protein, 321 aa, Escherichia coli str. K-12 substr. DH10B
MSDYQMFEVQVSQVEPLTEQVKRFTLVATDGKPLPAFTGGSHVIVQMSDGDNQYSNAYSLLSSPHDTSCYQIAVRLEENSRGGSRFLHQQVKVGDRLTISTPNNLFALIPSARKHLFIAGGIGITPFLSHMAELQHSDVDWQLHYCSRNPESCAFRDELVQHPQAEKVHLHHSSTGTRLELARLLADIEPGTHVYTCGPEALIEAVRSEAARLDIAADTLHFEQFAIEDKTGDAFTLVLARSGKEFVVPEEMTILQVIENNKAAKVECLCREGVCGTCETAILEGEADHRDQYFSDEERASQQSMLICCSRAKGKRLVLDL

SEQ ID NO: 7 - protein, 50 aa, Artificial sequence
  Synthetic
TTLSKSLAGAAKHERKAAKTLGIAVGIYLLCWLPFTIDTMVDSLLHFITP